European Patent Application EP 4 722 236 A1, published April 8, 2026. Title: 一种胰岛素衍生物及其应用. Applicant: 联邦生物科技（珠海横琴）有限公司. Application CN. The sequence listing filed with the application follows.

SEQUENCE LISTING (6 sequences)

SEQ ID NO: 1 - protein, 21 aa, synthetic construct
GIVEQCCTSICSLYQLENYCN

SEQ ID NO: 2 - protein, 30 aa, synthetic construct
FVNQHLCGSHLVEALYLVCGERGFFYTPKT

SEQ ID NO: 3 - protein, 21 aa, synthetic construct
GIVEQCCTSICSLEQLENYCN

SEQ ID NO: 4 - protein, 29 aa, synthetic construct
FVNQHLCGSHLVEALHLVCGERGFHYTPK

SEQ ID NO: 5 - protein, 21 aa, unidentified
GIVEQCCTSICSLEQLENYCN

SEQ ID NO: 6 - protein, 28 aa, synthetic construct
FVNQHLCGSHLVEALHLVCGERGFHYPK